European Patent Application EP 4 527 928 A1, published March 26, 2025. Title: Polynucleotides and uses in the treatment of Prader-Willi syndrome (PWS) and /or Prader-Willi like syndrome. Applicant: Université de Lorraine. The sequence listing filed with the application follows.

SEQUENCE LISTING (25 sequences)

SEQ ID NO: 1 - DNA, 20 bp, synthetic construct
  source 1..20: mol_type = other DNA
  variation 3: note = n is T or U
  variation 8: note = n is T or U
  variation 9: note = n is T or U
  variation 12: note = n is T or U
  variation 13: note = n is T or U
ggnggcannccnnggaaagg

SEQ ID NO: 2 - DNA, 20 bp, synthetic construct
  source 1..20: mol_type = other DNA; note = isolated polynucleotide
ggtggcattccttggaaagg

SEQ ID NO: 3 - RNA, 20 nt, synthetic construct
  source 1..20: mol_type = other RNA; note = isolated polynucleotide
ggtggcattccttggaaagg

SEQ ID NO: 4 - DNA, 21 bp, synthetic construct
  source 1..21: mol_type = other DNA; note = Gapdh RT qPCR primer
aacagcctcaagatcatcagc

SEQ ID NO: 5 - DNA, 20 bp, synthetic construct
  source 1..20: mol_type = other DNA; note = Gapdh RT qPCR primer
ggatgatgttctggagagcc

SEQ ID NO: 6 - DNA, 19 bp, synthetic construct
  source 1..19: mol_type = other DNA; note = Snord116 RT qPCR primer
tggatcgatgatgagtccc

SEQ ID NO: 7 - DNA, 20 bp, synthetic construct
  source 1..20: mol_type = other DNA; note = Snord116 RT qPCR primer
tggacctcagttccgatgag

SEQ ID NO: 8 - DNA, 20 bp, synthetic construct
  source 1..20: mol_type = other DNA; note = Dgkk RT qPCR primer
agaagccatcgctcatcagt

SEQ ID NO: 9 - DNA, 20 bp, synthetic construct
  source 1..20: mol_type = other DNA; note = Dgkk RT qPCR primer
tgaattttcggaggaagacg

SEQ ID NO: 10 - DNA, 16 bp, synthetic construct
  source 1..16: mol_type = other DNA; note = control oligonucleotide (G-CTR)
gctcccttcaatccaa

SEQ ID NO: 11 - DNA, 16 bp, synthetic construct
  source 1..16: mol_type = other DNA; note = oligonucleotide against endogenous snord116 (G-116)
tcactcattttgttca

SEQ ID NO: 12 - DNA, 19 bp, synthetic construct
  source 1..19: mol_type = other DNA; note = control oligonucleotide (SB-CTR)
taacacgtctatacgccca

SEQ ID NO: 13 - DNA, 16 bp, synthetic construct
  source 1..16: mol_type = other DNA; note = oligonucleotide SB1
aacattccttggaaaa

SEQ ID NO: 14 - DNA, 20 bp, synthetic construct
  source 1..20: mol_type = other DNA; note = primer for mouse Gapdh
ggcaaattcaacggcacagt

SEQ ID NO: 15 - DNA, 20 bp, synthetic construct
  source 1..20: mol_type = other DNA; note = primer for mouse Gapdh
gggtctcgctcctggaagat

SEQ ID NO: 16 - DNA, 20 bp, synthetic construct
  source 1..20: mol_type = other DNA; note = primer for mouse snord116
ggatctatgatgattcccag

SEQ ID NO: 17 - DNA, 18 bp, synthetic construct
  source 1..18: mol_type = other DNA; note = primer for mouse snord116
ggacctcagttccgatga

SEQ ID NO: 18 - DNA, 20 bp, synthetic construct
  source 1..20: mol_type = other DNA; note = primer for mouse Dgkk
gtcacaagagctgcggtagt

SEQ ID NO: 19 - DNA, 20 bp, synthetic construct
  source 1..20: mol_type = other DNA; note = primer for mouse Dgkk
cttggaaaaccgcttctggc

SEQ ID NO: 20 - DNA, 20 bp, synthetic construct
  source 1..20: mol_type = other DNA; note = primer for mouse Nlgn3
gcccgaaagcccaacaagaa

SEQ ID NO: 21 - DNA, 20 bp, synthetic construct
  source 1..20: mol_type = other DNA; note = primer for mouse Nlgn3
gctaagtcctcgccctgttt

SEQ ID NO: 22 - DNA, 20 bp, synthetic construct
  source 1..20: mol_type = other DNA; note = primer for mouse Rsbn1l
atgcgacagatcagcttggt

SEQ ID NO: 23 - DNA, 20 bp, synthetic construct
  source 1..20: mol_type = other DNA; note = primer for mouse Rsbn1l
ttctcctggacgtacccaca

SEQ ID NO: 24 - DNA, 20 bp, synthetic construct
  source 1..20: mol_type = other DNA; note = primer for mouse Nhlh2
ccgagctccgcaaactacta

SEQ ID NO: 25 - DNA, 20 bp, synthetic construct
  source 1..20: mol_type = other DNA; note = primer for mouse Nhlh2
atggccaagcgcagaatctc